European Patent Application EP 4 759 940 A1, published June 17, 2026. Title: 아고넛 단백질과 인공 핵산 회로를 이용한 표적 핵산 서열 검출 기술. Applicant: 한국생명공학연구원. Application KR. The sequence listing filed with the application follows.

SEQUENCE LISTING (39 sequences)

SEQ ID NO: 1 - DNA, 17 bp, synthetic construct
  source 1..17: mol_type = other DNA
  misc_binding 1: bound_moiety = the modification of phosphate group at 5'end.
tatcactgtattgcacg

SEQ ID NO: 2 - DNA, 17 bp, synthetic construct
  source 1..17: mol_type = other DNA
  misc_binding 1: bound_moiety = the modification of phosphate group at 5'end.
caaattggcggcggcgt

SEQ ID NO: 3 - DNA, 24 bp, synthetic construct
  source 1..24: mol_type = other DNA
gcggcgttatcactgtaactaaat

SEQ ID NO: 4 - DNA, 24 bp, synthetic construct
  source 1..24: mol_type = other DNA
  misc_binding 1: bound_moiety = binding FAM
  misc_binding 24: bound_moiety = binding BHQ2
gcggcgttatcactgtaactaaat

SEQ ID NO: 5 - DNA, 24 bp, synthetic construct
  source 1..24: mol_type = other DNA
atttagttacagtgataacgccgc

SEQ ID NO: 6 - DNA, 24 bp, synthetic construct
  source 1..24: mol_type = other DNA
  misc_binding 1: bound_moiety = binding BHQ2
  misc_binding 24: bound_moiety = binding FAM
atttagttacagtgataacgccgc

SEQ ID NO: 7 - DNA, 20 bp, synthetic construct
  source 1..20: mol_type = other DNA
ggttctgtggtcacccatct

SEQ ID NO: 8 - DNA, 20 bp, synthetic construct
  source 1..20: mol_type = other DNA
tccagacggaacgtggtatc

SEQ ID NO: 9 - DNA, 62 bp, Klebsiella pneumoniae
  source 1..62: mol_type = genomic DNA
ggtggcggagctgtccgcggccgccgtgcaatacagtgataacgccgccgccaatttgttgc

SEQ ID NO: 10 - DNA, 62 bp, synthetic construct
  source 1..62: mol_type = other DNA
gcaacaaattggcggcggcgttatcactgtattgcacggcggccgcggacagctccgccacc

SEQ ID NO: 11 - DNA, 17 bp, synthetic construct
  source 1..17: mol_type = other DNA
  misc_binding 1: bound_moiety = the modification of phosphate group at 5'end.
taacttttcagtatctt

SEQ ID NO: 12 - DNA, 17 bp, synthetic construct
  source 1..17: mol_type = other DNA
  misc_binding 1: bound_moiety = the modification of phosphate group at 5'end.
tccacaaaccaagtgac

SEQ ID NO: 13 - DNA, 24 bp, synthetic construct
  source 1..24: mol_type = other DNA
  misc_binding 1: bound_moiety = binding FAM
  misc_binding 24: bound_moiety = binding BHQ2
aagtgactaacttttcaactaaat

SEQ ID NO: 14 - DNA, 24 bp, synthetic construct
  source 1..24: mol_type = other DNA
atttagttgaaaagttagtcactt

SEQ ID NO: 15 - DNA, 20 bp, synthetic construct
  source 1..20: mol_type = other DNA
cctaaacatggcttggtggt

SEQ ID NO: 16 - DNA, 20 bp, synthetic construct
  source 1..20: mol_type = other DNA
gcatacgtggggatagatcg

SEQ ID NO: 17 - DNA, 64 bp, Klebsiella pneumoniae
  source 1..64: mol_type = genomic DNA
ctaattgacactccatttacggctaaagatactgaaaagttagtcacttggtttgtggagcgtg

SEQ ID NO: 18 - DNA, 64 bp, synthetic construct
  source 1..64: mol_type = other DNA
cacgctccacaaaccaagtgactaacttttcagtatctttagccgtaaatggagtgtcaattag

SEQ ID NO: 19 - DNA, 17 bp, synthetic construct
  source 1..17: mol_type = other DNA
taaactactaataactt

SEQ ID NO: 20 - DNA, 17 bp, synthetic construct
  source 1..17: mol_type = other DNA
gcggtcatgtagaccaa

SEQ ID NO: 21 - DNA, 24 bp, synthetic construct
  source 1..24: mol_type = other DNA
agaccaataaactactaactaaat

SEQ ID NO: 22 - DNA, 24 bp, synthetic construct
  source 1..24: mol_type = other DNA
atttagttagtagtttattggtct

SEQ ID NO: 23 - DNA, 17 bp, synthetic construct
  source 1..17: mol_type = other DNA
tagtagtttattggtct

SEQ ID NO: 24 - DNA, 64 bp, synthetic construct
  source 1..64: mol_type = other DNA
atgttaaaagttattagtagtttattggtctacatgaccgcgtctgtcatggctgtcgcaagtc

SEQ ID NO: 25 - DNA, 64 bp, synthetic construct
  source 1..64: mol_type = other DNA
gacttgcgacagccatgacagacgcggtcatgtagaccaataaactactaataacttttaacat

SEQ ID NO: 26 - DNA, 17 bp, synthetic construct
  source 1..17: mol_type = other DNA
taagtcgcaatccccgc

SEQ ID NO: 27 - DNA, 17 bp, synthetic construct
  source 1..17: mol_type = other DNA
tcgacaacgcattggca

SEQ ID NO: 28 - DNA, 24 bp, synthetic construct
  source 1..24: mol_type = other DNA
attggcataagtcgcaaactaaat

SEQ ID NO: 29 - DNA, 24 bp, synthetic construct
  source 1..24: mol_type = other DNA
atttagtttgcgacttatgccaat

SEQ ID NO: 30 - DNA, 17 bp, synthetic construct
  source 1..17: mol_type = other DNA
ttgcgacttatgccaat

SEQ ID NO: 31 - DNA, 64 bp, synthetic construct
  source 1..64: mol_type = other DNA
ggtatggacgcgctgcatgcggcggggattgcgacttatgccaatgcgttgtcgaaccagcttg

SEQ ID NO: 32 - DNA, 64 bp, synthetic construct
  source 1..64: mol_type = other DNA
caagctggttcgacaacgcattggcataagtcgcaatccccgccgcatgcagcgcgtccatacc

SEQ ID NO: 33 - DNA, 17 bp, synthetic construct
  source 1..17: mol_type = other DNA
tttcttaaaaagctgat

SEQ ID NO: 34 - DNA, 17 bp, synthetic construct
  source 1..17: mol_type = other DNA
acttattgtgatacagc

SEQ ID NO: 35 - DNA, 24 bp, synthetic construct
  source 1..24: mol_type = other DNA
atacagctttcttaaaaactaaat

SEQ ID NO: 36 - DNA, 24 bp, synthetic construct
  source 1..24: mol_type = other DNA
atttagtttttaagaaagctgtat

SEQ ID NO: 37 - DNA, 17 bp, synthetic construct
  source 1..17: mol_type = other DNA
ttttaagaaagctgtat

SEQ ID NO: 38 - DNA, 64 bp, synthetic construct
  source 1..64: mol_type = other DNA
attcgaatttcggccacggagcaaatcagctttttaagaaagctgtatcacaataagttacacg

SEQ ID NO: 39 - DNA, 64 bp, synthetic construct
  source 1..64: mol_type = other DNA
cgtgtaacttattgtgatacagctttcttaaaaagctgatttgctccgtggccgaaattcgaat